European Patent Application EP 4 176 870 A1, published May 10, 2023. Title: Extracellular vesicles or composition thereof for use as a medicament, such as for the treatment of ocular surface disorders. Applicant: HOPITAL FONDATION ADOLPHE DE ROTHSCHILD. The sequence listing filed with the application follows.

SEQUENCE LISTING (6 sequences)

SEQ ID NO: 1 - protein, 422 aa, Homo sapiens [sequence omitted]

SEQ ID NO: 2 - DNA, 1269 bp, Homo sapiens
atgcagaacagtcacagcggagtgaatcagctcggtggtgtctttgtcaacgggcggccactgccggactccacccggcagaagattgtagagctagctcacagcggggcccggccgtgcgacatttcccgaattctgcaggtgtccaacggatgtgtgagtaaaattctgggcaggtattacgagactggctccatcagacccagggcaatcggtggtagtaaaccgagagtagcgactccagaagttgtaagcaaaatagcccagtataagcgggagtgcccgtccatctttgcttgggaaatccgagacagattactgtccgagggggtctgtaccaacgataacataccaagcgtgtcatcaataaacagagttcttcgcaacctggctagcgaaaagcaacagatgggcgcagacggcatgtatgataaactaaggatgttgaacgggcagaccggaagctggggcacccgccctggttggtatccggggacttcggtgccagggcaacctacgcaagatggctgccagcaacaggaaggagggggagagaataccaactccatcagttccaacggagaagattcagatgaggctcaaatgcgacttcagctgaagcggaagctgcaaagaaatagaacatcctttacccaagagcaaattgaggccctggagaaagagtttgagagaacccattatccagatgtgtttgcccgagaaagactagcagccaaaatagatctacctgaagcaagaatacaggtatggttttctaatcgaagggccaaatggagaagagaagaaaaactgaggaatcagagaagacaggccagcaacacacctagtcatattcctatcagcagtagtttcagcaccagtgtctaccaaccaattccacaacccaccacaccggtttcctccttcacatctggctccatgttgggccgaacagacacagccctcacaaacacctacagcgctctgccgcctatgcccagcttcaccatggcaaataacctgcctatgcaacccccagtccccagccagacctcctcatactcctgcatgctgcccaccagcccttcggtgaatgggcggagttatgatacctacacccccccacatatgcagacacacatgaacagtcagccaatgggcacctcgggcaccacttcaacaggactcatttcccctggtgtgtcagttccagttcaagttcccggaagtgaacctgatatgtctcaatactggccaagattacagtaa

SEQ ID NO: 3 - protein, 436 aa, Homo sapiens
MQNSHSGVNQLGGVFVNGRPLPDSTRQKIVELAHSGARPCDISRILQTHADAKVQVLDNQNVSNGCVSKILGRYYETGSIRPRAIGGSKPRVATPEVVSKIAQYKRECPSIFAWEIRDRLLSEGVCTNDNIPSVSSINRVLRNLASEKQQMGADGMYDKLRMLNGQTGSWGTRPGWYPGTSVPGQPTQDGCQQQEGGGENTNSISSNGEDSDEAQMRLQLKRKLQRNRTSFTQEQIEALEKEFERTHYPDVFARERLAAKIDLPEARIQVWFSNRRAKWRREEKLRNQRRQASNTPSHIPISSSFSTSVYQPIPQPTTPVSSFTSGSMLGRTDTALTNTYSALPPMPSFTMANNLPMQPPVPSQTSSYSCMLPTSPSVNGRSYDTYTPPHMQTHMNSQPMGTSGTTSTGLISPGVSVPVQVPGSEPDMSQYWPRLQ

SEQ ID NO: 4 - DNA, 1311 bp, Homo sapiens
atgcagaacagtcacagcggagtgaatcagctcggtggtgtctttgtcaacgggcggccactgccggactccacccggcagaagattgtagagctagctcacagcggggcccggccgtgcgacatttcccgaattctgcagacccatgcagatgcaaaagtccaagtgctggacaatcaaaacgtgtccaacggatgtgtgagtaaaattctgggcaggtattacgagactggctccatcagacccagggcaatcggtggtagtaaaccgagagtagcgactccagaagttgtaagcaaaatagcccagtataagcgggagtgcccgtccatctttgcttgggaaatccgagacagattactgtccgagggggtctgtaccaacgataacataccaagcgtgtcatcaataaacagagttcttcgcaacctggctagcgaaaagcaacagatgggcgcagacggcatgtatgataaactaaggatgttgaacgggcagaccggaagctggggcacccgccctggttggtatccggggacttcggtgccagggcaacctacgcaagatggctgccagcaacaggaaggagggggagagaataccaactccatcagttccaacggagaagattcagatgaggctcaaatgcgacttcagctgaagcggaagctgcaaagaaatagaacatcctttacccaagagcaaattgaggccctggagaaagagtttgagagaacccattatccagatgtgtttgcccgagaaagactagcagccaaaatagatctacctgaagcaagaatacaggtatggttttctaatcgaagggccaaatggagaagagaagaaaaactgaggaatcagagaagacaggccagcaacacacctagtcatattcctatcagcagtagtttcagcaccagtgtctaccaaccaattccacaacccaccacaccggtttcctccttcacatctggctccatgttgggccgaacagacacagccctcacaaacacctacagcgctctgccgcctatgcccagcttcaccatggcaaataacctgcctatgcaacccccagtccccagccagacctcctcatactcctgcatgctgcccaccagcccttcggtgaatgggcggagttatgatacctacacccccccacatatgcagacacacatgaacagtcagccaatgggcacctcgggcaccacttcaacaggactcatttcccctggtgtgtcagttccagttcaagttcccggaagtgaacctgatatgtctcaatactggccaagattacagtaa

SEQ ID NO: 5 - protein, 2944 aa, Homo sapiens
MTLRLLVAALCAGILAEAPRVRAQHRERVTCTRLYAADIVFLLDGSSSIGRSNFREVRSFLEGLVLPFSGAASAQGVRFATVQYSDDPRTEFGLDALGSGGDVIRAIRELSYKGGNTRTGAAILHVADHVFLPQLARPGVPKVCILITDGKSQDLVDTAAQRLKGQGVKLFAVGIKNADPEELKRVASQPTSDFFFFVNDFSILRTLLPLVSRRVCTTAGGVPVTRPPDDSTSAPRDLVLSEPSSQSLRVQWTAASGPVTGYKVQYTPLTGLGQPLPSERQEVNVPAGETSVRLRGLRPLTEYQVTVIALYANSIGEAVSGTARTTALEGPELTIQNTTAHSLLVAWRSVPGATGYRVTWRVLSGGPTQQQELGPGQGSVLLRDLEPGTDYEVTVSTLFGRSVGPATSLMARTDASVEQTLRPVILGPTSILLSWNLVPEARGYRLEWRRETGLEPPQKVVLPSDVTRYQLDGLQPGTEYRLTLYTLLEGHEVATPATVVPTGPELPVSPVTDLQATELPGQRVRVSWSPVPGATQYRIIVRSTQGVERTLVLPGSQTAFDLDDVQAGLSYTVRVSARVGPREGSASVLTVRREPETPLAVPGLRVVVSDATRVRVAWGPVPGASGFRISWSTGSGPESSQTLPPDSTATDITGLQPGTTYQVAVSVLRGREEGPAAVIVARTDPLGPVRTVHVTQASSSSVTITWTRVPGATGYRVSWHSAHGPEKSQLVSGEATVAELDGLEPDTEYTVHVRAHVAGVDGPPASVVVRTAPEPVGRVSRLQILNASSDVLRITWVGVTGATAYRLAWGRSEGGPMRHQILPGNTDSAEIRGLEGGVSYSVRVTALVGDREGTPVSIVVTTPPEAPPALGTLHVVQRGEHSLRLRWEPVPRAQGFLLHWQPEGGQEQSRVLGPELSSYHLDGLEPATQYRVRLSVLGPAGEGPSAEVTARTESPRVPSIELRVVDTSIDSVTLAWTPVSRASSYILSWRPLRGPGQEVPGSPQTLPGISSSQRVTGLEPGVSYIFSLTPVLDGVRGPEASVTQTPVCPRGLADVVFLPHATQDNAHRAEATRRVLERLVLALGPLGPQAVQVGLLSYSHRPSPLFPLNGSHDLGIILQRIRDMPYMDPSGNNLGTAVVTAHRYMLAPDAPGRRQHVPGVMVLLVDEPLRGDIFSPIREAQASGLNVVMLGMAGADPEQLRRLAPGMDSVQTFFAVDDGPSLDQAVSGLATALCQASFTTQPRPEPCPVYCPKGQKGEPGEMGLRGQVGPPGDPGLPGRTGAPGPQGPPGSATAKGERGFPGADGRPGSPGRAGNPGTPGAPGLKGSPGLPGPRGDPGERGPRGPKGEPGAPGQVIGGEGPGLPGRKGDPGPSGPPGPRGPLGDPGPRGPPGLPGTAMKGDKGDRGERGPPGPGEGGIAPGEPGLPGLPGSPGPQGPVGPPGKKGEKGDSEDGAPGLPGQPGSPGEQGPRGPPGAIGPKGDRGFPGPLGEAGEKGERGPPGPAGSRGLPGVAGRPGAKGPEGPPGPTGRQGEKGEPGRPGDPAVVGPAVAGPKGEKGDVGPAGPRGATGVQGERGPPGLVLPGDPGPKGDPGDRGPIGLTGRAGPPGDSGPPGEKGDPGRPGPPGPVGPRGRDGEVGEKGDEGPPGDPGLPGKAGERGLRGAPGVRGPVGEKGDQGDPGEDGRNGSPGSSGPKGDRGEPGPPGPPGRLVDTGPGAREKGEPGDRGQEGPRGPKGDPGLPGAPGERGIEGFRGPPGPQGDPGVRGPAGEKGDRGPPGLDGRSGLDGKPGAAGPSGPNGAAGKAGDPGRDGLPGLRGEQGLPGPSGPPGLPGKPGEDGKPGLNGKNGEPGDPGEDGRKGEKGDSGASGREGRDGPKGERGAPGILGPQGPPGLPGPVGPPGQGFPGVPGGTGPKGDRGETGSKGEQGLPGERGLRGEPGSVPNVDRLLETAGIKASALREIVETWDESSGSFLPVPERRRGPKGDSGEQGPPGKEGPIGFPGERGLKGDRGDPGPQGPPGLALGERGPPGPSGLAGEPGKPGIPGLPGRAGGVGEAGRPGERGERGEKGERGEQGRDGPPGLPGTPGPPGPPGPKVSVDEPGPGLSGEQGPPGLKGAKGEPGSNGDQGPKGDRGVPGIKGDRGEPGPRGQDGNPGLPGERGMAGPEGKPGLQGPRGPPGPVGGHGDPGPPGAPGLAGPAGPQGPSGLKGEPGETGPPGRGLTGPTGAVGLPGPPGPSGLVGPQGSPGLPGQVGETGKPGAPGRDGASGKDGDRGSPGVPGSPGLPGPVGPKGEPGPTGAPGQAVVGLPGAKGEKGAPGGLAGDLVGEPGAKGDRGLPGPRGEKGEAGRAGEPGDPGEDGQKGAPGPKGFKGDPGVGVPGSPGPPGPPGVKGDLGLPGLPGAPGVVGFPGQTGPRGEMGQPGPSGERGLAGPPGREGIPGPLGPPGPPGSVGPPGASGLKGDKGDPGVGLPGPRGERGEPGIRGEDGRPGQEGPRGLTGPPGSRGERGEKGDVGSAGLKGDKGDSAVILGPPGPRGAKGDMGERGPRGLDGDKGPRGDNGDPGDKGSKGEPGDKGSAGLPGLRGLLGPQGQPGAAGIPGDPGSPGKDGVPGIRGEKGDVGFMGPRGLKGERGVKGACGLDGEKGDKGEAGPPGRPGLAGHKGEMGEPGVPGQSGAPGKEGLIGPKGDRGFDGQPGPKGDQGEKGERGTPGIGGFPGPSGNDGSAGPPGPPGSVGPRGPEGLQGQKGERGPPGERVVGAPGVPGAPGERGEQGRPGPAGPRGEKGEAALTEDDIRGFVRQEMSQHCACQGQFIASGSRPLPSYAADTAGSQLHAVPVLRVSHAEEEERVPPEDDEYSEYSEYSVEEYQDPEAPWDSDDPCSLPLDEGSCTAYTLRWYHRAVTGSTEACHPFVYGGCGGNANRFGTREACERRCPPRVVQSQGTGTAQD

SEQ ID NO: 6 - DNA, 8835 bp, Homo sapiens
atgacgctgcggcttctggtggccgcgctctgcgccgggatcctggcagaggcgccccgagtgcgagcccagcacagggagagagtgacctgcacgcgcctttacgccgctgacattgtgttcttactggatggctcctcatccattggccgcagcaatttccgcgaggtccgcagctttctcgaagggctggtgctgcctttctctggagcagccagtgcacagggtgtgcgctttgccacagtgcagtacagcgatgacccacggacagagttcggcctggatgcacttggctctgggggtgatgtgatccgcgccatccgtgagcttagctacaaggggggcaacactcgcacaggggctgcaattctccatgtggctgaccatgtcttcctgccccagctggcccgacctggtgtccccaaggtctgcatcctgatcacagacgggaagtcccaggacctggtggacacagctgcccaaaggctgaaggggcagggggtcaagctatttgctgtggggatcaagaatgctgaccctgaggagctgaagcgagttgcctcacagcccaccagtgacttcttcttcttcgtcaatgacttcagcatcttgaggacactactgcccctcgtttcccggagagtgtgcacgactgctggtggcgtgcctgtgacccgacctccggatgactcgacctctgctccacgagacctggtgctgtctgagccaagcagccaatccttgagagtacagtggacagcggccagtggccctgtgactggctacaaggtccagtacactcctctgacggggctgggacagccactgccgagtgagcggcaggaggtgaacgtcccagctggtgagaccagtgtgcggctgcggggtctccggccactgaccgagtaccaagtgactgtgattgccctctacgccaacagcatcggggaggctgtgagcgggacagctcggaccactgccctagaagggccggaactgaccatccagaataccacagcccacagcctcctggtggcctggcggagtgtgccaggtgccactggctaccgtgtgacatggcgggtcctcagtggtgggcccacacagcagcaggagctgggccctgggcagggttcagtgttgctgcgtgacttggagcctggcacggactatgaggtgaccgtgagcaccctatttggccgcagtgtggggcccgccacttccctgatggctcgcactgacgcttctgttgagcagaccctgcgcccggtcatcctgggccccacatccatcctcctttcctggaacttggtgcctgaggcccgtggctaccggttggaatggcggcgtgagactggcttggagccaccgcagaaggtggtactgccctctgatgtgacccgctaccagttggatgggctgcagccgggcactgagtaccgcctcacactctacactctgctggagggccacgaggtggccacccctgcaaccgtggttcccactggaccagagctgcctgtgagccctgtaacagacctgcaagccaccgagctgcccgggcagcgggtgcgagtgtcctggagcccagtccctggtgccacccagtaccgcatcattgtgcgcagcacccagggggttgagcggaccctggtgcttcctgggagtcagacagcattcgacttggatgacgttcaggctgggcttagctacactgtgcgggtgtctgctcgagtgggtccccgtgagggcagtgccagtgtcctcactgtccgccgggagccggaaactccacttgctgttccagggctgcgggttgtggtgtcagatgcaacgcgagtgagggtggcctggggacccgtccctggagccagtggatttcggattagctggagcacaggcagtggtccggagtccagccagacactgcccccagactctactgccacagacatcacagggctgcagcctggaaccacctaccaggtggctgtgtcggtactgcgaggcagagaggagggccctgctgcagtcatcgtggctcgaacggacccactgggcccagtgaggacggtccatgtgactcaggccagcagctcatctgtcaccattacctggaccagggttcctggcgccacaggatacagggtttcctggcactcagcccacggcccagagaaatcccagttggtttctggggaggccacggtggctgagctggatggactggagccagatactgagtatacggtgcatgtgagggcccatgtggctggcgtggatgggccccctgcctctgtggttgtgaggactgcccctgagcctgtgggtcgtgtgtcgaggctgcagatcctcaatgcttccagcgacgttctacggatcacctgggtaggggtcactggagccacagcttacagactggcctggggccggagtgaaggcggccccatgaggcaccagatactcccaggaaacacagactctgcagagatccggggtctcgaaggtggagtcagctactcagtgcgagtgactgcacttgtcggggaccgcgagggcacacctgtctccattgttgtcactacgccgcctgaggctccgccagccctggggacgcttcacgtggtgcagcgcggggagcactcgctgaggctgcgctgggagccggtgcccagagcgcagggcttccttctgcactggcaacctgagggtggccaggaacagtcccgggtcctggggcccgagctcagcagctatcacctggacgggctggagccagcgacacagtaccgcgtgaggctgagtgtcctagggccagctggagaagggccctctgcagaggtgactgcgcgcactgagtcacctcgtgttccaagcattgaactacgtgtggtggacacctcgatcgactcggtgactttggcctggactccagtgtccagggcatccagctacatcctatcctggcggccactcagaggccctggccaggaagtgcctgggtccccgcagacacttccagggatctcaagctcccagcgggtgacagggctagagcctggcgtctcttacatcttctccctgacgcctgtcctggatggtgtgcggggtcctgaggcatctgtcacacagacgccagtgtgcccccgtggcctggcggatgtggtgttcctaccacatgccactcaagacaatgctcaccgtgcggaggctacgaggagggtcctggagcgtctggtgttggcacttgggcctcttgggccacaggcagttcaggttggcctgctgtcttacagtcatcggccctccccactgttcccactgaatggctcccatgaccttggcattatcttgcaaaggatccgtgacatgccctacatggacccaagtgggaacaacctgggcacagccgtggtcacagctcacagatacatgttggcaccagatgctcctgggcgccgccagcacgtaccaggggtgatggttctgctagtggatgaacccttgagaggtgacatattcagccccatccgtgaggcccaggcttctgggcttaatgtggtgatgttgggaatggctggagcggacccagagcagctgcgtcgcttggcgccgggtatggactctgtccagaccttcttcgccgtggatgatgggccaagcctggaccaggcagtcagtggtctggccacagccctgtgtcaggcatccttcactactcagccccggccagagccctgcccagtgtattgtccaaagggccagaagggggaacctggagagatgggcctgagaggacaagttgggcctcctggcgaccctggcctcccgggcaggaccggtgctcccggcccccaggggccccctggaagtgccactgccaagggcgagaggggcttccctggagcagatgggcgtccaggcagccctggccgcgccgggaatcctgggacccctggagcccctggcctaaagggctctccagggttgcctggccctcgtggggacccgggagagcgaggacctcgaggcccaaagggggagccgggggctcccggacaagtcatcggaggtgaaggacctgggcttcctgggcggaaaggggaccctggaccatcgggcccccctggacctcgtggaccactgggggacccaggaccccgtggccccccagggcttcctggaacagccatgaagggtgacaaaggcgatcgtggggagcggggtccccctggaccaggtgaaggtggcattgctcctggggagcctgggctgccgggtcttcccggaagccctggaccccaaggccccgttggcccccctggaaagaaaggagaaaaaggtgactctgaggatggagctccaggcctcccaggacaacctgggtctccgggtgagcagggcccacggggacctcctggagctattggccccaaaggtgaccggggctttccagggcccctgggtgaggctggagagaagggcgaacgtggacccccaggcccagcgggatcccgggggctgccaggggttgctggacgtcctggagccaagggtcctgaagggccaccaggacccactggccgccaaggagagaagggggagcctggtcgccctggggaccctgcagtggtgggacctgctgttgctggacccaaaggagaaaagggagatgtggggcccgctgggcccagaggagctaccggagtccaaggggaacggggcccacccggcttggttcttcctggagaccctggccccaagggagaccctggagaccggggtcccattggccttactggcagagcaggacccccaggtgactcagggcctcctggagagaagggagaccctgggcggcctggccccccaggacctgttggcccccgaggacgagatggtgaagttggagagaaaggtgacgagggtcctccgggtgacccgggtttgcctggaaaagcaggcgagcgtggccttcggggggcacctggagttcgggggcctgtgggtgaaaagggagaccagggagatcctggagaggatggacgaaatggcagccctggatcatctggacccaagggtgaccgtggggagccgggtcccccaggacccccgggacggctggtagacacaggacctggagccagagagaagggagagcctggggaccgcggacaagagggtcctcgagggcccaagggtgatcctggcctccctggagcccctggggaaaggggcattgaagggtttcggggacccccaggcccacagggggacccaggtgtccgaggcccagcaggagaaaagggtgaccggggtccccctgggctggatggccggagcggactggatgggaaaccaggagccgctgggccctctgggccgaatggtgctgcaggcaaagctggggacccagggagagacgggcttccaggcctccgtggagaacagggcctccctggcccctctggtccccctggattaccgggaaagccaggcgaggatggcaaacctggcctgaatggaaaaaacggagaacctggggaccctggagaagacgggaggaagggagagaaaggagattcaggcgcctctgggagagaaggtcgtgatggccccaagggtgagcgtggagctcctggtatccttggaccccaggggcctccaggcctcccagggccagtgggccctcctggccagggttttcctggtgtcccaggaggcacgggccccaagggtgaccgtggggagactggatccaaaggggagcagggcctccctggagagcgtggcctgcgaggagagcctggaagtgtgccgaatgtggatcggttgctggaaactgctggcatcaaggcatctgccctgcgggagatcgtggagacctgggatgagagctctggtagcttcctgcctgtgcccgaacggcgtcgaggccccaagggggactcaggcgaacagggccccccaggcaaggagggccccatcggctttcctggagaacgcgggctgaagggcgaccgtggagaccctggccctcaggggccacctggtctggcccttggggagaggggcccccccgggccttccggccttgccggggagcctggaaagcctggtattcccgggctcccaggcagggctgggggtgtgggagaggcaggaaggccaggagagaggggagaacggggagagaaaggagaacgtggagaacagggcagagatggccctcctggactccctggaacccctgggccccccggaccccctggccccaaggtgtctgtggatgagccaggtcctggactctctggagaacagggaccccctggactcaagggtgctaagggggagccgggcagcaatggtgaccaaggtcccaaaggagacaggggtgtgccaggcatcaaaggagaccggggagagcctggaccgaggggtcaggacggcaacccgggtctaccaggagagcgtggtatggctgggcctgaagggaagccgggtctgcagggtccaagaggcccccctggcccagtgggtggtcatggagaccctggaccacctggtgccccgggtcttgctggccctgcaggaccccaaggaccttctggcctgaagggggagcctggagagacaggacctccaggacggggcctgactggacctactggagctgtgggacttcctggaccccccggcccttcaggccttgtgggtccacaggggtctccaggtttgcctggacaagtgggggagacagggaagccgggagccccaggtcgagatggtgccagtggaaaagatggagacagagggagccctggtgtgccagggtcaccaggtctgcctggccctgtcggacctaaaggagaacctggccccacgggggcccctggacaggctgtggtcgggctccctggagcaaagggagagaagggagcccctggaggccttgctggagacctggtgggtgagccgggagccaaaggtgaccgaggactgccagggccgcgaggcgagaagggtgaagctggccgtgcaggggagcccggagaccctggggaagatggtcagaaaggggctccaggacccaaaggtttcaagggtgacccaggagtcggggtcccgggctcccctgggcctcctggccctccaggtgtgaagggagatctgggcctccctggcctgcccggtgctcctggtgttgttgggttcccgggtcagacaggccctcgaggagagatgggtcagccaggccctagtggagagcggggtctggcaggccccccagggagagaaggaatcccaggacccctggggccacctggaccaccggggtcagtgggaccacctggggcctctggactcaaaggagacaagggagaccctggagtagggctgcctgggccccgaggcgagcgtggggagccaggcatccggggtgaagatggccgccccggccaggagggaccccgaggactcacggggccccctggcagcaggggagagcgtggggagaagggtgatgttgggagtgcaggactaaagggtgacaagggagactcagctgtgatcctggggcctccaggcccacggggtgccaagggggacatgggtgaacgagggcctcggggcttggatggtgacaaaggacctcggggagacaatggggaccctggtgacaagggcagcaagggagagcctggtgacaagggctcagccgggttgccaggactgcgtggactcctgggaccccagggtcaacctggtgcagcagggatccctggtgacccgggatccccaggaaaggatggagtgcctggtatccgaggagaaaaaggagatgttggcttcatgggtccccggggcctcaagggtgaacggggagtgaagggagcctgtggccttgatggagagaagggagacaagggagaagctggtcccccaggccgccccgggctggcaggacacaaaggagagatgggggagcctggtgtgccgggccagtcgggggcccctggcaaggagggcctgatcggtcccaagggtgaccgaggctttgacgggcagccaggccccaagggtgaccagggcgagaaaggggagcggggaaccccaggaattgggggcttcccaggccccagtggaaatgatggctctgctggtcccccagggccacctggcagtgttggtcccagaggccccgaaggacttcagggccagaagggtgagcgaggtccccccggagagagagtggtgggggctcctggggtccctggagctcctggcgagagaggggagcaggggcggccagggcctgccggtcctcgaggcgagaagggagaagctgcactgacggaggatgacatccggggctttgtgcgccaagagatgagtcagcactgtgcctgccagggccagttcatcgcatctggatcacgacccctccctagttatgctgcagacactgccggctcccagctccatgctgtgcctgtgctccgcgtctctcatgcagaggaggaagagcgggtaccccctgaggatgatgagtactctgaatactccgagtattctgtggaggagtaccaggaccctgaagctccttgggatagtgatgacccctgttccctgccactggatgagggctcctgcactgcctacaccctgcgctggtaccatcgggctgtgacaggcagcacagaggcctgtcacccttttgtctatggtggctgtggagggaatgccaaccgttttgggacccgtgaggcctgcgagcgccgctgcccaccccgggtggtccagagccaggggacaggtactgcccaggactga